European Patent Specification EP 3 768 296 B1, published September 6, 2023. Title: SAP AND PEPTIDOMIMETICS FOR TREATMENT OF EYE DISEASE. Applicant: Arch Biosurgery, Inc. NORCHI, TERRENCE ELLIS-BEHNKE, RUTLEDGE. The sequence listing filed with the application follows.

SEQUENCE LISTING (445 sequences)

SEQ ID NO: 1 - protein, 16 aa, Artificial Sequence
  Synthetic Peptide
RADARADARADARADA

SEQ ID NO: 2 - protein, 16 aa, Artificial Sequence
  Synthetic Peptide
SGSGSGSGSGSGSGSG

SEQ ID NO: 3 - protein, 16 aa, Artificial Sequence
  Synthetic Peptide
SASASASASASASASA

SEQ ID NO: 4 - protein, 16 aa, Artificial Sequence
  Synthetic Peptide
SVSVSVSVSVSVSVSV

SEQ ID NO: 5 - protein, 16 aa, Artificial Sequence
  Synthetic Peptide
SLSLSLSLSLSLSLSL

SEQ ID NO: 6 - protein, 16 aa, Artificial Sequence
  Synthetic Peptide
SISISISISISISISI

SEQ ID NO: 7 - protein, 16 aa, Artificial Sequence
  Synthetic Peptide
SMSMSMSMSMSMSMSM

SEQ ID NO: 8 - protein, 16 aa, Artificial Sequence
  Synthetic Peptide
SFSFSFSFSFSFSFSF

SEQ ID NO: 9 - protein, 16 aa, Artificial Sequence
  Synthetic Peptide
SWSWSWSWSWSWSWSW

SEQ ID NO: 10 - protein, 16 aa, Artificial Sequence
  Synthetic Peptide
SPSPSPSPSPSPSPSP

SEQ ID NO: 11 - protein, 16 aa, Artificial Sequence
  Synthetic Peptide
TGTGTGTGTGTGTGTG

SEQ ID NO: 12 - protein, 16 aa, Artificial Sequence
  Synthetic Peptide
TATATATATATATATA

SEQ ID NO: 13 - protein, 16 aa, Artificial Sequence
  Synthetic Peptide
TVTVTVTVTVTVTVTV

SEQ ID NO: 14 - protein, 16 aa, Artificial Sequence
  Synthetic Peptide
TLTLTLTLTLTLTLTL

SEQ ID NO: 15 - protein, 16 aa, Artificial Sequence
  Synthetic Peptide
TITITITITITITITI

SEQ ID NO: 16 - protein, 16 aa, Artificial Sequence
  Synthetic Peptide
TMTMTMTMTMTMTMTM

SEQ ID NO: 17 - protein, 16 aa, Artificial Sequence
  Synthetic Peptide
TFTFTFTFTFTFTFTF

SEQ ID NO: 18 - protein, 16 aa, Artificial Sequence
  Synthetic Peptide
TWTWTWTWTWTWTWTW

SEQ ID NO: 19 - protein, 16 aa, Artificial Sequence
  Synthetic Peptide
TPTPTPTPTPTPTPTP

SEQ ID NO: 20 - protein, 16 aa, Artificial Sequence
  Synthetic Peptide
CGCGCGCGCGCGCGCG

SEQ ID NO: 21 - protein, 16 aa, Artificial Sequence
  Synthetic Peptide
CACACACACACACACA

SEQ ID NO: 22 - protein, 16 aa, Artificial Sequence
  Synthetic Peptide
CVCVCVCVCVCVCVCV

SEQ ID NO: 23 - protein, 16 aa, Artificial Sequence
  Synthetic Peptide
CLCLCLCLCLCLCLCL

SEQ ID NO: 24 - protein, 16 aa, Artificial Sequence
  Synthetic Peptide
CICICICICICICICI

SEQ ID NO: 25 - protein, 16 aa, Artificial Sequence
  Synthetic Peptide
CMCMCMCMCMCMCMCM

SEQ ID NO: 26 - protein, 16 aa, Artificial Sequence
  Synthetic Peptide
CFCFCFCFCFCFCFCF

SEQ ID NO: 27 - protein, 15 aa, Artificial Sequence
  Synthetic Peptide
CWCWCWCWCWCWCWC

SEQ ID NO: 28 - protein, 16 aa, Artificial Sequence
  Synthetic Peptide
CPCPCPCPCPCPCPCP

SEQ ID NO: 29 - protein, 16 aa, Artificial Sequence
  Synthetic Peptide
YGYGYGYGYGYGYGYG

SEQ ID NO: 30 - protein, 16 aa, Artificial Sequence
  Synthetic Peptide
YAYAYAYAYAYAYAYA

SEQ ID NO: 31 - protein, 16 aa, Artificial Sequence
  Synthetic Peptide
YVYVYVYVYVYVYVYV

SEQ ID NO: 32 - protein, 16 aa, Artificial Sequence
  Synthetic Peptide
YLYLYLYLYLYLYLYL

SEQ ID NO: 33 - protein, 16 aa, Artificial Sequence
  Synthetic Peptide
YIYIYIYIYIYIYIYI

SEQ ID NO: 34 - protein, 16 aa, Artificial Sequence
  Synthetic Peptide
YMYMYMYMYMYMYMYM

SEQ ID NO: 35 - protein, 16 aa, Artificial Sequence
  Synthetic Peptide
YFYFYFYFYFYFYFYF

SEQ ID NO: 36 - protein, 16 aa, Artificial Sequence
  Synthetic Peptide
YWYWYWYWYWYWYWYW

SEQ ID NO: 37 - protein, 16 aa, Artificial Sequence
  Synthetic Peptide
YPYPYPYPYPYPYPYP

SEQ ID NO: 38 - protein, 16 aa, Artificial Sequence
  Synthetic Peptide
NGNGNGNGNGNGNGNG

SEQ ID NO: 39 - protein, 16 aa, Artificial Sequence
  Synthetic Peptide
NANANANANANANANA

SEQ ID NO: 40 - protein, 16 aa, Artificial Sequence
  Synthetic Peptide
NVNVNVNVNVNVNVNV

SEQ ID NO: 41 - protein, 16 aa, Artificial Sequence
  Synthetic Peptide
NLNLNLNLNLNLNLNL

SEQ ID NO: 42 - protein, 16 aa, Artificial Sequence
  Synthetic Peptide
NINININININININI

SEQ ID NO: 43 - protein, 16 aa, Artificial Sequence
  Synthetic Peptide
NMNMNMNMNMNMNMNM

SEQ ID NO: 44 - protein, 16 aa, Artificial Sequence
  Synthetic Peptide
NFNFNFNFNFNFNFNF

SEQ ID NO: 45 - protein, 16 aa, Artificial Sequence
  Synthetic Peptide
NWNWNWNWNWNWNWNW

SEQ ID NO: 46 - protein, 16 aa, Artificial Sequence
  Synthetic Peptide
NPNPNPNPNPNPNPNP

SEQ ID NO: 47 - protein, 16 aa, Artificial Sequence
  Synthetic Peptide
QGQGQGQGQGQGQGQG

SEQ ID NO: 48 - protein, 16 aa, Artificial Sequence
  Synthetic Peptide
QAQAQAQAQAQAQAQA

SEQ ID NO: 49 - protein, 16 aa, Artificial Sequence
  Synthetic Peptide
QVQVQVQVQVQVQVQV

SEQ ID NO: 50 - protein, 16 aa, Artificial Sequence
  Synthetic Peptide
QLQLQLQLQLQLQLQL

SEQ ID NO: 51 - protein, 16 aa, Artificial Sequence
  Synthetic Peptide
QIQIQIQIQIQIQIQI

SEQ ID NO: 52 - protein, 16 aa, Artificial Sequence
  Synthetic Peptide
QMQMQMQMQMQMQMQM

SEQ ID NO: 53 - protein, 16 aa, Artificial Sequence
  Synthetic Peptide
QFQFQFQFQFQFQFQF

SEQ ID NO: 54 - protein, 16 aa, Artificial Sequence
  Synthetic Peptide
QWQWQWQWQWQWQWQW

SEQ ID NO: 55 - protein, 16 aa, Artificial Sequence
  Synthetic Peptide
QPQPQPQPQPQPQPQP

SEQ ID NO: 56 - protein, 16 aa, Artificial Sequence
  Synthetic Peptide
AEAKAEAKAEAKAEAK

SEQ ID NO: 57 - protein, 4 aa, Artificial Sequence
  Synthetic Peptide
RADA

SEQ ID NO: 58 - protein, 16 aa, Artificial Sequence
  Synthetic Peptide
RAEARAEARAEARAEA

SEQ ID NO: 59 - protein, 16 aa, Artificial Sequence
  Synthetic Peptide
KADAKADAKADAKADA

SEQ ID NO: 60 - protein, 13 aa, Artificial Sequence
  Synthetic Peptide
ARADARADARADA

SEQ ID NO: 61 - protein, 20 aa, Artificial Sequence
  Synthetic Peptide
RADARADARADARADARADA

SEQ ID NO: 62 - protein, 21 aa, Artificial Sequence
  Synthetic Peptide
ARADARADARADARADARADA

SEQ ID NO: 63 - protein, 17 aa, Artificial Sequence
  Synthetic Peptide
ARADARADARADARADA

SEQ ID NO: 64 - protein, 16 aa, Artificial Sequence
  Synthetic Peptide
RLDLRLDLRLDLRLDL

SEQ ID NO: 65 - protein, 4 aa, Artificial Sequence
  Synthetic Peptide
RLDL

SEQ ID NO: 66 - protein, 6 aa, Artificial Sequence
  Synthetic Peptide
RLDLRL

SEQ ID NO: 67 - protein, 6 aa, Artificial Sequence
  Synthetic Peptide
RADARA

SEQ ID NO: 68 - protein, 6 aa, Artificial Sequence
  Synthetic Peptide
LRLDLR

SEQ ID NO: 69 - protein, 13 aa, Artificial Sequence
  Synthetic Peptide
IEIKIEIKIEIKI

SEQ ID NO: 70 - protein, 16 aa, Artificial Sequence
  Synthetic Peptide
IEIKIEIKIEIKIEIK

SEQ ID NO: 71 - protein, 17 aa, Artificial Sequence
  Synthetic Peptide
IEIKIEIKIEIKIEIKI

SEQ ID NO: 72 - protein, 20 aa, Artificial Sequence
  Synthetic Peptide
IEIKIEIKIEIKIEIKIEIK

SEQ ID NO: 73 - protein, 21 aa, Artificial Sequence
  Synthetic Peptide
IEIKIEIKIEIKIEIKIEIKI

SEQ ID NO: 74 - protein, 12 aa, Artificial Sequence
  Synthetic Peptide
IEIKIEIKIEIK

SEQ ID NO: 75 - protein, 16 aa, Artificial Sequence
  Synthetic Peptide
EIKIEIKIEIKIEIKI

SEQ ID NO: 76 - protein, 16 aa, Artificial Sequence
  Synthetic Peptide
EAKAEAKAEAKAEAKA

SEQ ID NO: 77 - protein, 4 aa, Artificial Sequence
  Synthetic Peptide
EAKA

SEQ ID NO: 78 - protein, 10 aa, Artificial Sequence
  Synthetic Peptide
EAKAEAKAEA

SEQ ID NO: 79 - protein, 20 aa, Artificial Sequence
  Synthetic Peptide
EAKAEAKAEAKAEAKAEAKA

SEQ ID NO: 80 - protein, 17 aa, Artificial Sequence
  Synthetic Peptide
AEAKAEAKAEAKAEAKA

SEQ ID NO: 81 - protein, 13 aa, Artificial Sequence
  Synthetic Peptide
AEAKAEAKAEAKA

SEQ ID NO: 82 - protein, 18 aa, Artificial Sequence
  Synthetic Peptide
RADARADARADARADLRA

SEQ ID NO: 83 - protein, 16 aa, Artificial Sequence
  Synthetic Peptide
  MISC_FEATURE (1)..(1): D-arginine
  MISC_FEATURE (2)..(2): D-alanine
  MISC_FEATURE (3)..(3): D-aspartic acid
  MISC_FEATURE (4)..(4): D-alanine
  MISC_FEATURE (5)..(5): D-arginine
  MISC_FEATURE (6)..(6): D-alanine
  MISC_FEATURE (7)..(7): D-aspartic acid
  MISC_FEATURE (8)..(8): D-alanine
  MISC_FEATURE (9)..(9): D-arginine
  MISC_FEATURE (10)..(10): D-alanine
  MISC_FEATURE (11)..(11): D-aspartic acid
  MISC_FEATURE (12)..(12): D-alanine
  MISC_FEATURE (13)..(13): D-arginine
  MISC_FEATURE (14)..(14): D-alanine
  MISC_FEATURE (15)..(15): D-aspartic acid
  MISC_FEATURE (16)..(16): D-alanine
RADARADARADARADA

SEQ ID NO: 84 - protein, 12 aa, Artificial Sequence
  Synthetic Peptide
  MISC_FEATURE (1)..(1): D-arginine
  MISC_FEATURE (2)..(2): D-alanine
  MISC_FEATURE (3)..(3): D-aspartic acid
  MISC_FEATURE (4)..(4): D-alanine
  MISC_FEATURE (5)..(5): D-arginine
  MISC_FEATURE (6)..(6): D-alanine
  MISC_FEATURE (7)..(7): D-aspartic acid
  MISC_FEATURE (8)..(8): D-alanine
  MISC_FEATURE (9)..(9): D-arginine
  MISC_FEATURE (10)..(10): D-alanine
  MISC_FEATURE (11)..(11): D-aspartic acid
  MISC_FEATURE (12)..(12): D-alanine
RADARADARADA

SEQ ID NO: 85 - protein, 12 aa, Artificial Sequence
  Synthetic Peptide
  MISC_FEATURE (1)..(1): D-glutamic acid
  MISC_FEATURE (2)..(2): D-alanine
  MISC_FEATURE (3)..(3): D-lysine
  MISC_FEATURE (4)..(4): D-alanine
  MISC_FEATURE (5)..(5): D-glutamic acid
  MISC_FEATURE (6)..(6): D-alanine
  MISC_FEATURE (7)..(7): D-lysine
  MISC_FEATURE (8)..(8): D-alanine
  MISC_FEATURE (9)..(9): D-glutamic acid
  MISC_FEATURE (10)..(10): D-alanine
  MISC_FEATURE (11)..(11): D-lysine
  MISC_FEATURE (12)..(12): D-alanine
EAKAEAKAEAKA

SEQ ID NO: 86 - protein, 4 aa, Artificial Sequence
  Synthetic Peptide
  MISC_FEATURE (1)..(1): D-glutamic acid
  MISC_FEATURE (2)..(2): D-alanine
  MISC_FEATURE (3)..(3): D-lysine
  MISC_FEATURE (4)..(4): D-alanine
EAKA

SEQ ID NO: 87 - protein, 4 aa, Artificial Sequence
  Synthetic Peptide
  MISC_FEATURE (1)..(1): D-arginine
  MISC_FEATURE (2)..(2): D-alanine
  MISC_FEATURE (3)..(3): D-aspartic acid
  MISC_FEATURE (4)..(4): D-alanine
RADA

SEQ ID NO: 88 - protein, 8 aa, Artificial Sequence
  Synthetic Peptide
RADARADA

SEQ ID NO: 89 - protein, 16 aa, Artificial Sequence
  Synthetic Peptide
EARAEARAEARAEARA

SEQ ID NO: 90 - protein, 12 aa, Artificial Sequence
  Synthetic Peptide
EARAEARAEARA

SEQ ID NO: 91 - protein, 9 aa, Artificial Sequence
  Synthetic Peptide
EARAEARAE

SEQ ID NO: 92 - protein, 4 aa, Artificial Sequence
  Synthetic Peptide
EARA

SEQ ID NO: 93 - protein, 9 aa, Artificial Sequence
  Synthetic Peptide
  NH2 (9)..(9): C-terminal amine
CYIQNCPRG

SEQ ID NO: 94 - protein, 7 aa, Artificial Sequence
  Synthetic Peptide
  MISC_FEATURE (4)..(5): amino succinyl modification
  NH2 (7)..(7): C-terminal amine
YFQNPRG

SEQ ID NO: 95 - protein, 7 aa, Artificial Sequence
  Synthetic Peptide
  MISC_FEATURE (4)..(5): amino succinyl modification
  NH2 (7)..(7): C-terminal amine
YIQNPRG

SEQ ID NO: 96 - protein, 7 aa, Artificial Sequence
  Synthetic Peptide
  MISC_FEATURE (1)..(1): 3-mercaptopropionyl-D-Pyridylanine modification
  NH2 (7)..(7): C-terminal amine
FQNCPRG

SEQ ID NO: 97 - protein, 10 aa, Artificial Sequence
  Synthetic Peptide
  Xaa (1)..(1): Xaa = deamino penicillamine
  NH2 (10)..(10): C-terminal amine
XYFVNCPDRG

SEQ ID NO: 98 - protein, 8 aa, Artificial Sequence
  Synthetic Peptide
  MISC_FEATURE (1)..(1): 3-mercaptopropionyl modification
  NH2 (8)..(8): C-terminal amine
YFQNCPRG

SEQ ID NO: 99 - protein, 9 aa, Artificial Sequence
  Synthetic Peptide
  MISC_FEATURE (1)..(1): 3-mercaptopropionyl modification
  NH2 (9)..(9): C-terminal amine
YFQNCPDRG

SEQ ID NO: 100 - protein, 7 aa, Artificial Sequence
  Synthetic Peptide
  MISC_FEATURE (1)..(1): 3-mercaptopropionyl modification
YFQNCPK

SEQ ID NO: 101 - protein, 9 aa, Artificial Sequence
  Synthetic Peptide
  NH2 (9)..(9): C-terminal amine
CYFQNCPKG

SEQ ID NO: 102 - protein, 8 aa, Artificial Sequence
  Synthetic Peptide
CYFQNCPK

SEQ ID NO: 103 - protein, 9 aa, Artificial Sequence
  Synthetic Peptide
  MISC_FEATURE (1)..(1): 3-mercaptopropionyl modification
  NH2 (9)..(9): C-terminal amine
YFVNCPDRG

SEQ ID NO: 104 - protein, 9 aa, Artificial Sequence
  Synthetic Peptide
  Xaa (8)..(8): Xaa = ornithine
  NH2 (9)..(9): C-terminal amine
CFIQNCPXG

SEQ ID NO: 105 - protein, 9 aa, Artificial Sequence
  Synthetic Peptide
  MISC_FEATURE (1)..(1): pyridoxamine phosphate modification
  MISC_FEATURE (2)..(2): ethoxy modification
  Xaa (8)..(8): Xaa = citrulline
  NH2 (9)..(9): C-terminal amine
DYFVNCPXG

SEQ ID NO: 106 - protein, 8 aa, Artificial Sequence
  Synthetic Peptide
  MISC_FEATURE (1)..(1): pyridoxamine phosphate modification
  MISC_FEATURE (1)..(1): ethoxy modification
  NH2 (8)..(8): C-terminal amine
YFVNCPRG

SEQ ID NO: 107 - protein, 8 aa, Artificial Sequence
  Synthetic Peptide
  MISC_FEATURE (1)..(1): pyridoxamine phosphate modification
  Me (1)..(1): Methylation
  NH2 (8)..(8): C-terminal amine
YFQNCPRG

SEQ ID NO: 108 - protein, 8 aa, Artificial Sequence
  Synthetic Peptide
  MISC_FEATURE (1)..(1): pyridoxamine phosphate modification
  Me (1)..(1): methylation
  Xaa (7)..(7): Xaa = ornithine
  NH2 (8)..(8): C-terminal amine
YIQNCPXG

SEQ ID NO: 109 - protein, 7 aa, Artificial Sequence
  Synthetic Peptide
GDRGDSP

SEQ ID NO: 110 - protein, 11 aa, Artificial Sequence
  Synthetic Peptide
GDRGDSPASSK

SEQ ID NO: 111 - protein, 10 aa, Artificial Sequence
  Synthetic Peptide
  Xaa (2)..(2): Xaa = penicillamine
GXGRGDSPCA

SEQ ID NO: 112 - protein, 6 aa, Artificial Sequence
  Synthetic Peptide
GRADSP

SEQ ID NO: 113 - protein, 7 aa, Artificial Sequence
  Synthetic Peptide
GRGDDSP

SEQ ID NO: 114 - protein, 6 aa, Artificial Sequence
  Synthetic Peptide
GRGDNP

SEQ ID NO: 115 - protein, 5 aa, Artificial Sequence
  Synthetic Peptide
GRGDS

SEQ ID NO: 116 - protein, 6 aa, Artificial Sequence
  Synthetic Peptide
GRGDSP

SEQ ID NO: 117 - protein, 7 aa, Artificial Sequence
  Synthetic Peptide
GRGDSPC

SEQ ID NO: 118 - protein, 7 aa, Artificial Sequence
  Synthetic Peptide
GRGDSPK

SEQ ID NO: 119 - protein, 6 aa, Artificial Sequence
  Synthetic Peptide
GRGDTP

SEQ ID NO: 120 - protein, 5 aa, Artificial Sequence
  Synthetic Peptide
GRGES

SEQ ID NO: 121 - protein, 6 aa, Artificial Sequence
  Synthetic Peptide
GRGESP

SEQ ID NO: 122 - protein, 6 aa, Artificial Sequence
  Synthetic Peptide
GRGETP

SEQ ID NO: 123 - protein, 4 aa, Artificial Sequence
  Synthetic Peptide
KGDS

SEQ ID NO: 124 - protein, 6 aa, Artificial Sequence
  Synthetic Peptide
GAVSTA

SEQ ID NO: 125 - protein, 6 aa, Artificial Sequence
  Synthetic Peptide
WTVPTA

SEQ ID NO: 126 - protein, 11 aa, Artificial Sequence
  Synthetic Peptide
TDVNGDGRHDL

SEQ ID NO: 127 - protein, 4 aa, Artificial Sequence
  Synthetic Peptide
REDV

SEQ ID NO: 128 - protein, 4 aa, Artificial Sequence
  Synthetic Peptide
RGDC

SEQ ID NO: 129 - protein, 4 aa, Artificial Sequence
  Synthetic Peptide
RGDS

SEQ ID NO: 130 - protein, 10 aa, Artificial Sequence
  Synthetic Peptide
RGDSPASSKP

SEQ ID NO: 131 - protein, 4 aa, Artificial Sequence
  Synthetic Peptide
RGDT

SEQ ID NO: 132 - protein, 4 aa, Artificial Sequence
  Synthetic Peptide
RGDV

SEQ ID NO: 133 - protein, 4 aa, Artificial Sequence
  Synthetic Peptide
RGES

SEQ ID NO: 134 - protein, 4 aa, Artificial Sequence
  Synthetic Peptide
SDGR

SEQ ID NO: 135 - protein, 5 aa, Artificial Sequence
  Synthetic Peptide
SDGRG

SEQ ID NO: 136 - protein, 5 aa, Artificial Sequence
  Synthetic Peptide
YRGDS

SEQ ID NO: 137 - protein, 14 aa, Artificial Sequence [sequence omitted]

SEQ ID NO: 138 - protein, 17 aa, Artificial Sequence
  Synthetic Peptide
YADSGEGDFLAEGGGVR

SEQ ID NO: 139 - protein, 14 aa, Artificial Sequence
  Synthetic Peptide
  MISC_FEATURE (1)..(1): Glp modification
GVNDNEEGFFSARY

SEQ ID NO: 140 - protein, 8 aa, Artificial Sequence
  Synthetic Peptide
  MISC_FEATURE (1)..(1): Cy5.5 modification
RARARARA

SEQ ID NO: 141 - protein, 7 aa, Artificial Sequence
  Synthetic Peptide
MSCRAMM

SEQ ID NO: 142 - protein, 16 aa, Artificial Sequence
  Synthetic Peptide
GGGGGDGDGDGDGDGD

SEQ ID NO: 143 - protein, 16 aa, Artificial Sequence
  Synthetic Peptide
GGGGGEGEGEGEGEGE

SEQ ID NO: 144 - protein, 16 aa, Artificial Sequence
  Synthetic Peptide
GGGGGKGKGKGKGKGK

SEQ ID NO: 145 - protein, 16 aa, Artificial Sequence
  Synthetic Peptide
GGGGGRGRGRGRGRGR

SEQ ID NO: 146 - protein, 16 aa, Artificial Sequence
  Synthetic Peptide
GGGGGHGHGHGHGHGH

SEQ ID NO: 147 - protein, 16 aa, Artificial Sequence
  Synthetic Peptide
AAAAADADADADADAD

SEQ ID NO: 148 - protein, 16 aa, Artificial Sequence
  Synthetic Peptide
AAAAAEAEAEAEAEAE

SEQ ID NO: 149 - protein, 16 aa, Artificial Sequence
  Synthetic Peptide
AAAAAKAKAKAKAKAK

SEQ ID NO: 150 - protein, 16 aa, Artificial Sequence
  Synthetic Peptide
AAAAARARARARARAR

SEQ ID NO: 151 - protein, 16 aa, Artificial Sequence
  Synthetic Peptide
AAAAAHAHAHAHAHAH

SEQ ID NO: 152 - protein, 16 aa, Artificial Sequence
  Synthetic Peptide
VVVVVDVDVDVDVDVD

SEQ ID NO: 153 - protein, 16 aa, Artificial Sequence
  Synthetic Peptide
VVVVVEVEVEVEVEVE

SEQ ID NO: 154 - protein, 16 aa, Artificial Sequence
  Synthetic Peptide
VVVVVKVKVKVKVKVK

SEQ ID NO: 155 - protein, 16 aa, Artificial Sequence
  Synthetic Peptide
VVVVVRVRVRVRVRVR

SEQ ID NO: 156 - protein, 16 aa, Artificial Sequence
  Synthetic Peptide
VVVVVHVHVHVHVHVH

SEQ ID NO: 157 - protein, 16 aa, Artificial Sequence
  Synthetic Peptide
LLLLLDLDLDLDLDLD

SEQ ID NO: 158 - protein, 16 aa, Artificial Sequence
  Synthetic Peptide
LLLLLELELELELELE

SEQ ID NO: 159 - protein, 16 aa, Artificial Sequence
  Synthetic Peptide
LLLLLKLKLKLKLKLK

SEQ ID NO: 160 - protein, 16 aa, Artificial Sequence
  Synthetic Peptide
LLLLLRLRLRLRLRLR

SEQ ID NO: 161 - protein, 16 aa, Artificial Sequence
  Synthetic Peptide
LLLLLHLHLHLHLHLH

SEQ ID NO: 162 - protein, 16 aa, Artificial Sequence
  Synthetic Peptide
IIIIIDIDIDIDIDID

SEQ ID NO: 163 - protein, 16 aa, Artificial Sequence
  Synthetic Peptide
IIIIIEIEIEIEIEIE

SEQ ID NO: 164 - protein, 16 aa, Artificial Sequence
  Synthetic Peptide
IIIIIKIKIKIKIKIK

SEQ ID NO: 165 - protein, 16 aa, Artificial Sequence
  Synthetic Peptide
IIIIIRIRIRIRIRIR

SEQ ID NO: 166 - protein, 16 aa, Artificial Sequence
  Synthetic Peptide
IIIIIHIHIHIHIHIH

SEQ ID NO: 167 - protein, 16 aa, Artificial Sequence
  Synthetic Peptide
MMMMMDMDMDMDMDMD

SEQ ID NO: 168 - protein, 16 aa, Artificial Sequence
  Synthetic Peptide
MMMMMEMEMEMEMEME

SEQ ID NO: 169 - protein, 16 aa, Artificial Sequence
  Synthetic Peptide
MMMMMKMKMKMKMKMK

SEQ ID NO: 170 - protein, 16 aa, Artificial Sequence
  Synthetic Peptide
MMMMMRMRMRMRMRMR

SEQ ID NO: 171 - protein, 16 aa, Artificial Sequence
  Synthetic Peptide
MMMMMHMHMHMHMHMH

SEQ ID NO: 172 - protein, 16 aa, Artificial Sequence
  Synthetic Peptide
FFFFFDFDFDFDFDFD

SEQ ID NO: 173 - protein, 16 aa, Artificial Sequence
  Synthetic Peptide
FFFFFEFEFEFEFEFE

SEQ ID NO: 174 - protein, 16 aa, Artificial Sequence
  Synthetic Peptide
FFFFFKFKFKFKFKFK

SEQ ID NO: 175 - protein, 16 aa, Artificial Sequence
  Synthetic Peptide
FFFFFRFRFRFRFRFR

SEQ ID NO: 176 - protein, 16 aa, Artificial Sequence
  Synthetic Peptide
FFFFFHFHFHFHFHFH

SEQ ID NO: 177 - protein, 16 aa, Artificial Sequence
  Synthetic Peptide
WWWWWDWDWDWDWDWD

SEQ ID NO: 178 - protein, 16 aa, Artificial Sequence
  Synthetic Peptide
WWWWWEWEWEWEWEWE

SEQ ID NO: 179 - protein, 16 aa, Artificial Sequence
  Synthetic Peptide
WWWWWKWKWKWKWKWK

SEQ ID NO: 180 - protein, 16 aa, Artificial Sequence
  Synthetic Peptide
WWWWWRWRWRWRWRWR

SEQ ID NO: 181 - protein, 16 aa, Artificial Sequence
  Synthetic Peptide
WWWWWHWHWHWHWHWH

SEQ ID NO: 182 - protein, 16 aa, Artificial Sequence
  Synthetic Peptide
PPPPPDPDPDPDPDPD

SEQ ID NO: 183 - protein, 16 aa, Artificial Sequence
  Synthetic Peptide
PPPPPEPEPEPEPEPE

SEQ ID NO: 184 - protein, 16 aa, Artificial Sequence
  Synthetic Peptide
PPPPPKPKPKPKPKPK

SEQ ID NO: 185 - protein, 16 aa, Artificial Sequence
  Synthetic Peptide
PPPPPRPRPRPRPRPR

SEQ ID NO: 186 - protein, 16 aa, Artificial Sequence
  Synthetic Peptide
PPPPPHPHPHPHPHPH

SEQ ID NO: 187 - protein, 16 aa, Artificial Sequence
  Synthetic Peptide
AAAAARADARADARAD

SEQ ID NO: 188 - protein, 16 aa, Artificial Sequence
  Synthetic Peptide
AAAAARARADADARAR

SEQ ID NO: 189 - protein, 16 aa, Artificial Sequence
  Synthetic Peptide
AAAAAEAKAEAKAEAK

SEQ ID NO: 190 - protein, 16 aa, Artificial Sequence
  Synthetic Peptide
AAAAAEAEAKAKAEAE

SEQ ID NO: 191 - protein, 16 aa, Artificial Sequence
  Synthetic Peptide
AAAAARAEARAEARAE

SEQ ID NO: 192 - protein, 16 aa, Artificial Sequence
  Synthetic Peptide
AAAAARARAEAEARAE

SEQ ID NO: 193 - protein, 16 aa, Artificial Sequence
  Synthetic Peptide
AAAAAKADAKADAKAD

SEQ ID NO: 194 - protein, 16 aa, Artificial Sequence
  Synthetic Peptide
AAAAAEAHAEAHAEAH

SEQ ID NO: 195 - protein, 16 aa, Artificial Sequence
  Synthetic Peptide
AAAAAEAEAHAHAEAE

SEQ ID NO: 196 - protein, 16 aa, Artificial Sequence
  Synthetic Peptide
AAAAARARARARADAD

SEQ ID NO: 197 - protein, 16 aa, Artificial Sequence
  Synthetic Peptide
AAAAARARARADADAD

SEQ ID NO: 198 - protein, 16 aa, Artificial Sequence
  Synthetic Peptide
AAAAAHADAHADAHAD

SEQ ID NO: 199 - protein, 16 aa, Artificial Sequence
  Synthetic Peptide
AAAAAHADADAHADAD

SEQ ID NO: 200 - protein, 16 aa, Artificial Sequence
  Synthetic Peptide
AAAAAHAEAEAHAEAE

SEQ ID NO: 201 - protein, 16 aa, Artificial Sequence
  Synthetic Peptide
GGGGGRGDGRGDGRGD

SEQ ID NO: 202 - protein, 16 aa, Artificial Sequence
  Synthetic Peptide
GGGGGRGRGDGDGRGR

SEQ ID NO: 203 - protein, 16 aa, Artificial Sequence
  Synthetic Peptide
GGGGGEGKGEGKGEGK

SEQ ID NO: 204 - protein, 16 aa, Artificial Sequence
  Synthetic Peptide
GGGGGEGEGKGKGEGE

SEQ ID NO: 205 - protein, 16 aa, Artificial Sequence
  Synthetic Peptide
GGGGGRGEGRGEGRGE

SEQ ID NO: 206 - protein, 16 aa, Artificial Sequence
  Synthetic Peptide
GGGGGRGRGEGEGRGE

SEQ ID NO: 207 - protein, 16 aa, Artificial Sequence
  Synthetic Peptide
GGGGGKGDGKGDGKGD

SEQ ID NO: 208 - protein, 16 aa, Artificial Sequence
  Synthetic Peptide
GGGGGEGHGEGHGEGH

SEQ ID NO: 209 - protein, 16 aa, Artificial Sequence
  Synthetic Peptide
GGGGGEGEGHGHGEGE

SEQ ID NO: 210 - protein, 16 aa, Artificial Sequence
  Synthetic Peptide
GGGGGRGRGRGRGDGD

SEQ ID NO: 211 - protein, 16 aa, Artificial Sequence
  Synthetic Peptide
GGGGGRGRGRGDGDGD

SEQ ID NO: 212 - protein, 16 aa, Artificial Sequence
  Synthetic Peptide
GGGGGHGDGHGDGHGD

SEQ ID NO: 213 - protein, 16 aa, Artificial Sequence
  Synthetic Peptide
GGGGGHGDGDGHGDGD

SEQ ID NO: 214 - protein, 16 aa, Artificial Sequence
  Synthetic Peptide
GGGGGHGEGEGHGEGE

SEQ ID NO: 215 - protein, 16 aa, Artificial Sequence
  Synthetic Peptide
VVVVVRVDVRVDVRVD

SEQ ID NO: 216 - protein, 16 aa, Artificial Sequence
  Synthetic Peptide
VVVVVRVRVDVDVRVR

SEQ ID NO: 217 - protein, 16 aa, Artificial Sequence
  Synthetic Peptide
VVVVVEVKVEVKVEVK

SEQ ID NO: 218 - protein, 16 aa, Artificial Sequence
  Synthetic Peptide
VVVVVEVEVKVKVEVE

SEQ ID NO: 219 - protein, 16 aa, Artificial Sequence
  Synthetic Peptide
VVVVVRVEVRVEVRVE

SEQ ID NO: 220 - protein, 16 aa, Artificial Sequence
  Synthetic Peptide
VVVVVRVRVEVEVRVE

SEQ ID NO: 221 - protein, 16 aa, Artificial Sequence
  Synthetic Peptide
VVVVVKVDVKVDVKVD

SEQ ID NO: 222 - protein, 16 aa, Artificial Sequence
  Synthetic Peptide
VVVVVEVHVEVHVEVH

SEQ ID NO: 223 - protein, 16 aa, Artificial Sequence
  Synthetic Peptide
VVVVVEVEVHVHVEVE

SEQ ID NO: 224 - protein, 16 aa, Artificial Sequence
  Synthetic Peptide
VVVVVRVRVRVRVDVD

SEQ ID NO: 225 - protein, 16 aa, Artificial Sequence
  Synthetic Peptide
VVVVVRVRVRVDVDVD

SEQ ID NO: 226 - protein, 16 aa, Artificial Sequence
  Synthetic Peptide
VVVVVHVDVHVDVHVD

SEQ ID NO: 227 - protein, 16 aa, Artificial Sequence
  Synthetic Peptide
VVVVVHVDVDVHVDVD

SEQ ID NO: 228 - protein, 16 aa, Artificial Sequence
  Synthetic Peptide
VVVVVHVEVEVHVEVE

SEQ ID NO: 229 - protein, 16 aa, Artificial Sequence
  Synthetic Peptide
LLLLLRLDLRLDLRLD

SEQ ID NO: 230 - protein, 16 aa, Artificial Sequence
  Synthetic Peptide
LLLLLRLRLDLDLRLR

SEQ ID NO: 231 - protein, 16 aa, Artificial Sequence
  Synthetic Peptide
LLLLLELKLELKLELK

SEQ ID NO: 232 - protein, 16 aa, Artificial Sequence
  Synthetic Peptide
LLLLLELELKLKLELE

SEQ ID NO: 233 - protein, 16 aa, Artificial Sequence
  Synthetic Peptide
LLLLLRLELRLELRLE

SEQ ID NO: 234 - protein, 16 aa, Artificial Sequence
  Synthetic Peptide
LLLLLRLRLELELRLE

SEQ ID NO: 235 - protein, 16 aa, Artificial Sequence
  Synthetic Peptide
LLLLLKLDLKLDLKLD

SEQ ID NO: 236 - protein, 16 aa, Artificial Sequence
  Synthetic Peptide
LLLLLELHLELHLELH

SEQ ID NO: 237 - protein, 16 aa, Artificial Sequence
  Synthetic Peptide
LLLLLELELHLHLELE

SEQ ID NO: 238 - protein, 16 aa, Artificial Sequence
  Synthetic Peptide
LLLLLRLRLRLRLDLD

SEQ ID NO: 239 - protein, 16 aa, Artificial Sequence
  Synthetic Peptide
LLLLLRLRLRLDLDLD

SEQ ID NO: 240 - protein, 16 aa, Artificial Sequence
  Synthetic Peptide
LLLLLHLDLHLDLHLD

SEQ ID NO: 241 - protein, 16 aa, Artificial Sequence
  Synthetic Peptide
LLLLLHLDLDLHLDLD

SEQ ID NO: 242 - protein, 16 aa, Artificial Sequence
  Synthetic Peptide
LLLLLHLELELHLELE

SEQ ID NO: 243 - protein, 16 aa, Artificial Sequence
  Synthetic Peptide
IIIIIRIDIRIDIRID

SEQ ID NO: 244 - protein, 16 aa, Artificial Sequence
  Synthetic Peptide
IIIIIRIRIDIDIRIR

SEQ ID NO: 245 - protein, 16 aa, Artificial Sequence
  Synthetic Peptide
IIIIIEIKIEIKIEIK

SEQ ID NO: 246 - protein, 16 aa, Artificial Sequence
  Synthetic Peptide
IIIIIEIEIKIKIEIE

SEQ ID NO: 247 - protein, 16 aa, Artificial Sequence
  Synthetic Peptide
IIIIIRIEIRIEIRIE

SEQ ID NO: 248 - protein, 16 aa, Artificial Sequence
  Synthetic Peptide
IIIIIRIRIEIEIRIE

SEQ ID NO: 249 - protein, 16 aa, Artificial Sequence
  Synthetic Peptide
IIIIIKIDIKIDIKID

SEQ ID NO: 250 - protein, 16 aa, Artificial Sequence
  Synthetic Peptide
IIIIIEIHIEIHIEIH

SEQ ID NO: 251 - protein, 16 aa, Artificial Sequence
  Synthetic Peptide
IIIIIEIEIHIHIEIE

SEQ ID NO: 252 - protein, 16 aa, Artificial Sequence
  Synthetic Peptide
IIIIIRIRIRIRIDID

SEQ ID NO: 253 - protein, 16 aa, Artificial Sequence
  Synthetic Peptide
IIIIIRIRIRIDIDID

SEQ ID NO: 254 - protein, 16 aa, Artificial Sequence
  Synthetic Peptide
IIIIIHIDIHIDIHID

SEQ ID NO: 255 - protein, 16 aa, Artificial Sequence
  Synthetic Peptide
IIIIIHIDIDIHIDID

SEQ ID NO: 256 - protein, 16 aa, Artificial Sequence
  Synthetic Peptide
IIIIIHIEIEIHIEIE

SEQ ID NO: 257 - protein, 16 aa, Artificial Sequence
  Synthetic Peptide
MMMMMRMDMRMDMRMD

SEQ ID NO: 258 - protein, 16 aa, Artificial Sequence
  Synthetic Peptide
MMMMMRMRMDMDMRMR

SEQ ID NO: 259 - protein, 16 aa, Artificial Sequence
  Synthetic Peptide
MMMMMEMKMEMKMEMK

SEQ ID NO: 260 - protein, 16 aa, Artificial Sequence
  Synthetic Peptide
MMMMMEMEMKMKMEME

SEQ ID NO: 261 - protein, 16 aa, Artificial Sequence
  Synthetic Peptide
MMMMMRMEMRMEMRME

SEQ ID NO: 262 - protein, 16 aa, Artificial Sequence
  Synthetic Peptide
MMMMMRMRMEMEMRME

SEQ ID NO: 263 - protein, 16 aa, Artificial Sequence
  Synthetic Peptide
MMMMMKMDMKMDMKMD

SEQ ID NO: 264 - protein, 16 aa, Artificial Sequence
  Synthetic Peptide
MMMMMEMHMEMHMEMH

SEQ ID NO: 265 - protein, 16 aa, Artificial Sequence
  Synthetic Peptide
MMMMMEMEMHMHMEME

SEQ ID NO: 266 - protein, 16 aa, Artificial Sequence
  Synthetic Peptide
MMMMMRMRMRMRMDMD

SEQ ID NO: 267 - protein, 16 aa, Artificial Sequence
  Synthetic Peptide
MMMMMRMRMRMDMDMD

SEQ ID NO: 268 - protein, 16 aa, Artificial Sequence
  Synthetic Peptide
MMMMMHMDMHMDMHMD

SEQ ID NO: 269 - protein, 16 aa, Artificial Sequence
  Synthetic Peptide
MMMMMHMDMDMHMDMD

SEQ ID NO: 270 - protein, 16 aa, Artificial Sequence
  Synthetic Peptide
MMMMMHMEMEMHMEME

SEQ ID NO: 271 - protein, 16 aa, Artificial Sequence
  Synthetic Peptide
FFFFFRFDFRFDFRFD

SEQ ID NO: 272 - protein, 16 aa, Artificial Sequence
  Synthetic Peptide
FFFFFRFRFDFDFRFR

SEQ ID NO: 273 - protein, 16 aa, Artificial Sequence
  Synthetic Peptide
FFFFFEFKFEFKFEFK

SEQ ID NO: 274 - protein, 16 aa, Artificial Sequence
  Synthetic Peptide
FFFFFEFEFKFKFEFE

SEQ ID NO: 275 - protein, 16 aa, Artificial Sequence
  Synthetic Peptide
FFFFFRFEFRFEFRFE

SEQ ID NO: 276 - protein, 16 aa, Artificial Sequence
  Synthetic Peptide
FFFFFRFRFEFEFRFE

SEQ ID NO: 277 - protein, 16 aa, Artificial Sequence
  Synthetic Peptide
FFFFFKFDFKFDFKFD

SEQ ID NO: 278 - protein, 16 aa, Artificial Sequence
  Synthetic Peptide
FFFFFEFHFEFHFEFH

SEQ ID NO: 279 - protein, 16 aa, Artificial Sequence
  Synthetic Peptide
FFFFFEFEFHFHFEFE

SEQ ID NO: 280 - protein, 16 aa, Artificial Sequence
  Synthetic Peptide
FFFFFRFRFRFRFDFD

SEQ ID NO: 281 - protein, 16 aa, Artificial Sequence
  Synthetic Peptide
FFFFFRFRFRFDFDFD

SEQ ID NO: 282 - protein, 16 aa, Artificial Sequence
  Synthetic Peptide
FFFFFHFDFHFDFHFD

SEQ ID NO: 283 - protein, 16 aa, Artificial Sequence
  Synthetic Peptide
FFFFFHFDFDFHFDFD

SEQ ID NO: 284 - protein, 16 aa, Artificial Sequence
  Synthetic Peptide
FFFFFHFEFEFHFEFE

SEQ ID NO: 285 - protein, 16 aa, Artificial Sequence
  Synthetic Peptide
WWWWWRWDWRWDWRWD

SEQ ID NO: 286 - protein, 16 aa, Artificial Sequence
  Synthetic Peptide
WWWWWRWRWDWDWRWR

SEQ ID NO: 287 - protein, 16 aa, Artificial Sequence
  Synthetic Peptide
WWWWWEWKWEWKWEWK

SEQ ID NO: 288 - protein, 16 aa, Artificial Sequence
  Synthetic Peptide
WWWWWEWEWKWKWEWE

SEQ ID NO: 289 - protein, 16 aa, Artificial Sequence
  Synthetic Peptide
WWWWWRWEWRWEWRWE

SEQ ID NO: 290 - protein, 16 aa, Artificial Sequence
  Synthetic Peptide
WWWWWRWRWEWEWRWE

SEQ ID NO: 291 - protein, 16 aa, Artificial Sequence
  Synthetic Peptide
WWWWWKWDWKWDWKWD

SEQ ID NO: 292 - protein, 16 aa, Artificial Sequence
  Synthetic Peptide
WWWWWEWHWEWHWEWH

SEQ ID NO: 293 - protein, 16 aa, Artificial Sequence
  Synthetic Peptide
WWWWWEWEWHWHWEWE

SEQ ID NO: 294 - protein, 16 aa, Artificial Sequence
  Synthetic Peptide
WWWWWRWRWRWRWDWD

SEQ ID NO: 295 - protein, 16 aa, Artificial Sequence
  Synthetic Peptide
WWWWWRWRWRWDWDWD

SEQ ID NO: 296 - protein, 16 aa, Artificial Sequence
  Synthetic Peptide
WWWWWHWDWHWDWHWD

SEQ ID NO: 297 - protein, 16 aa, Artificial Sequence
  Synthetic Peptide
WWWWWHWDWDWHWDWD

SEQ ID NO: 298 - protein, 16 aa, Artificial Sequence
  Synthetic Peptide
WWWWWHWEWEWHWEWE

SEQ ID NO: 299 - protein, 16 aa, Artificial Sequence
  Synthetic Peptide
PPPPPRPDPRPDPRPD

SEQ ID NO: 300 - protein, 16 aa, Artificial Sequence
  Synthetic Peptide
PPPPPRPRPDPDPRPR

SEQ ID NO: 301 - protein, 16 aa, Artificial Sequence
  Synthetic Peptide
PPPPPEPKPEPKPEPK

SEQ ID NO: 302 - protein, 16 aa, Artificial Sequence
  Synthetic Peptide
PPPPPEPEPKPKPEPE

SEQ ID NO: 303 - protein, 16 aa, Artificial Sequence
  Synthetic Peptide
PPPPPRPEPRPEPRPE

SEQ ID NO: 304 - protein, 16 aa, Artificial Sequence
  Synthetic Peptide
PPPPPRPRPEPEPRPE

SEQ ID NO: 305 - protein, 16 aa, Artificial Sequence
  Synthetic Peptide
PPPPPKPDPKPDPKPD

SEQ ID NO: 306 - protein, 16 aa, Artificial Sequence
  Synthetic Peptide
PPPPPEPHPEPHPEPH

SEQ ID NO: 307 - protein, 16 aa, Artificial Sequence
  Synthetic Peptide
PPPPPEPEPHPHPEPE

SEQ ID NO: 308 - protein, 16 aa, Artificial Sequence
  Synthetic Peptide
PPPPPRPRPRPRPDPD

SEQ ID NO: 309 - protein, 16 aa, Artificial Sequence
  Synthetic Peptide
PPPPPRPRPRPDPDPD

SEQ ID NO: 310 - protein, 16 aa, Artificial Sequence
  Synthetic Peptide
PPPPPHPDPHPDPHPD

SEQ ID NO: 311 - protein, 16 aa, Artificial Sequence
  Synthetic Peptide
PPPPPHPDPDPHPDPD

SEQ ID NO: 312 - protein, 16 aa, Artificial Sequence
  Synthetic Peptide
PPPPPHPEPEPHPEPE

SEQ ID NO: 313 - protein, 16 aa, Artificial Sequence
  Synthetic Peptide
SSSSSRSDSRSDSRSD

SEQ ID NO: 314 - protein, 16 aa, Artificial Sequence
  Synthetic Peptide
SSSSSRSRSDSDSRSR

SEQ ID NO: 315 - protein, 16 aa, Artificial Sequence
  Synthetic Peptide
SSSSSESKSESKSESK

SEQ ID NO: 316 - protein, 16 aa, Artificial Sequence
  Synthetic Peptide
SSSSSESESKSKSESE

SEQ ID NO: 317 - protein, 16 aa, Artificial Sequence
  Synthetic Peptide
SSSSSRSESRSESRSE

SEQ ID NO: 318 - protein, 16 aa, Artificial Sequence
  Synthetic Peptide
SSSSSRSRSESESRSE

SEQ ID NO: 319 - protein, 16 aa, Artificial Sequence
  Synthetic Peptide
SSSSSKSDSKSDSKSD

SEQ ID NO: 320 - protein, 16 aa, Artificial Sequence
  Synthetic Peptide
SSSSSESHSESHSESH

SEQ ID NO: 321 - protein, 16 aa, Artificial Sequence
  Synthetic Peptide
SSSSSESESHSHSESE

SEQ ID NO: 322 - protein, 16 aa, Artificial Sequence
  Synthetic Peptide
SSSSSRSRSRSRSRSR

SEQ ID NO: 323 - protein, 16 aa, Artificial Sequence
  Synthetic Peptide
SSSSSRSRSRSRSDSD

SEQ ID NO: 324 - protein, 16 aa, Artificial Sequence
  Synthetic Peptide
SSSSSRSRSRSDSDSD

SEQ ID NO: 325 - protein, 16 aa, Artificial Sequence
  Synthetic Peptide
SSSSSHSDSHSDSHSD

SEQ ID NO: 326 - protein, 16 aa, Artificial Sequence
  Synthetic Peptide
SSSSSHSHSHSHSHSH

SEQ ID NO: 327 - protein, 16 aa, Artificial Sequence
  Synthetic Peptide
SSSSSHSDSDSHSDSD

SEQ ID NO: 328 - protein, 16 aa, Artificial Sequence
  Synthetic Peptide
SSSSSHSESESHSESE

SEQ ID NO: 329 - protein, 16 aa, Artificial Sequence
  Synthetic Peptide
TTTTTRTDTRTDTRTD

SEQ ID NO: 330 - protein, 16 aa, Artificial Sequence
  Synthetic Peptide
TTTTTRTRTDTDTRTR

SEQ ID NO: 331 - protein, 16 aa, Artificial Sequence
  Synthetic Peptide
TTTTTETKTETKTETK

SEQ ID NO: 332 - protein, 16 aa, Artificial Sequence
  Synthetic Peptide
TTTTTETETKTKTETE

SEQ ID NO: 333 - protein, 16 aa, Artificial Sequence
  Synthetic Peptide
TTTTTRTETRTETRTE

SEQ ID NO: 334 - protein, 16 aa, Artificial Sequence
  Synthetic Peptide
TTTTTRTRTETETRTE

SEQ ID NO: 335 - protein, 16 aa, Artificial Sequence
  Synthetic Peptide
TTTTTKTDTKTDTKTD

SEQ ID NO: 336 - protein, 16 aa, Artificial Sequence
  Synthetic Peptide
TTTTTETHTETHTETH

SEQ ID NO: 337 - protein, 16 aa, Artificial Sequence
  Synthetic Peptide
TTTTTETETHTHTETE

SEQ ID NO: 338 - protein, 16 aa, Artificial Sequence
  Synthetic Peptide
TTTTTRTRTRTRTRTR

SEQ ID NO: 339 - protein, 16 aa, Artificial Sequence
  Synthetic Peptide
TTTTTRTRTRTRTDTD

SEQ ID NO: 340 - protein, 16 aa, Artificial Sequence
  Synthetic Peptide
TTTTTRTRTRTDTDTD

SEQ ID NO: 341 - protein, 16 aa, Artificial Sequence
  Synthetic Peptide
TTTTTHTDTHTDTHTD

SEQ ID NO: 342 - protein, 16 aa, Artificial Sequence
  Synthetic Peptide
TTTTTHTHTHTHTHTH

SEQ ID NO: 343 - protein, 16 aa, Artificial Sequence
  Synthetic Peptide
TTTTTHTDTDTHTDTD

SEQ ID NO: 344 - protein, 16 aa, Artificial Sequence
  Synthetic Peptide
TTTTTHTETETHTETE

SEQ ID NO: 345 - protein, 16 aa, Artificial Sequence
  Synthetic Peptide
CCCCCRCDCRCDCRCD

SEQ ID NO: 346 - protein, 16 aa, Artificial Sequence
  Synthetic Peptide
CCCCCRCRCDCDCRCR

SEQ ID NO: 347 - protein, 16 aa, Artificial Sequence
  Synthetic Peptide
CCCCCECKCECKCECK

SEQ ID NO: 348 - protein, 16 aa, Artificial Sequence
  Synthetic Peptide
CCCCCECECKCKCECE

SEQ ID NO: 349 - protein, 16 aa, Artificial Sequence
  Synthetic Peptide
CCCCCRCECRCECRCE

SEQ ID NO: 350 - protein, 16 aa, Artificial Sequence
  Synthetic Peptide
CCCCCRCRCECECRCE

SEQ ID NO: 351 - protein, 16 aa, Artificial Sequence
  Synthetic Peptide
CCCCCKCDCKCDCKCD

SEQ ID NO: 352 - protein, 16 aa, Artificial Sequence
  Synthetic Peptide
CCCCCECHCECHCECH

SEQ ID NO: 353 - protein, 16 aa, Artificial Sequence
  Synthetic Peptide
CCCCCECECHCHCECE

SEQ ID NO: 354 - protein, 16 aa, Artificial Sequence
  Synthetic Peptide
CCCCCRCRCRCRCRCR

SEQ ID NO: 355 - protein, 16 aa, Artificial Sequence
  Synthetic Peptide
CCCCCRCRCRCRCDCD

SEQ ID NO: 356 - protein, 16 aa, Artificial Sequence
  Synthetic Peptide
CCCCCRCRCRCDCDCD

SEQ ID NO: 357 - protein, 16 aa, Artificial Sequence
  Synthetic Peptide
CCCCCHCDCHCDCHCD

SEQ ID NO: 358 - protein, 16 aa, Artificial Sequence
  Synthetic Peptide
CCCCCHCHCHCHCHCH

SEQ ID NO: 359 - protein, 16 aa, Artificial Sequence
  Synthetic Peptide
CCCCCHCDCDCHCDCD

SEQ ID NO: 360 - protein, 16 aa, Artificial Sequence
  Synthetic Peptide
CCCCCHCECECHCECE

SEQ ID NO: 361 - protein, 16 aa, Artificial Sequence
  Synthetic Peptide
YYYYYRYDYRYDYRYD

SEQ ID NO: 362 - protein, 16 aa, Artificial Sequence
  Synthetic Peptide
YYYYYRYRYDYDYRYR

SEQ ID NO: 363 - protein, 16 aa, Artificial Sequence
  Synthetic Peptide
YYYYYEYKYEYKYEYK

SEQ ID NO: 364 - protein, 16 aa, Artificial Sequence
  Synthetic Peptide
YYYYYEYEYKYKYEYE

SEQ ID NO: 365 - protein, 16 aa, Artificial Sequence
  Synthetic Peptide
YYYYYRYEYRYEYRYE

SEQ ID NO: 366 - protein, 16 aa, Artificial Sequence
  Synthetic Peptide
YYYYYRYRYEYEYRYE

SEQ ID NO: 367 - protein, 16 aa, Artificial Sequence
  Synthetic Peptide
YYYYYKYDYKYDYKYD

SEQ ID NO: 368 - protein, 16 aa, Artificial Sequence
  Synthetic Peptide
YYYYYEYHYEYHYEYH

SEQ ID NO: 369 - protein, 16 aa, Artificial Sequence
  Synthetic Peptide
YYYYYEYEYHYHYEYE

SEQ ID NO: 370 - protein, 16 aa, Artificial Sequence
  Synthetic Peptide
YYYYYRYRYRYRYRYR

SEQ ID NO: 371 - protein, 16 aa, Artificial Sequence
  Synthetic Peptide
YYYYYRYRYRYRYDYD

SEQ ID NO: 372 - protein, 16 aa, Artificial Sequence
  Synthetic Peptide
YYYYYRYRYRYDYDYD

SEQ ID NO: 373 - protein, 16 aa, Artificial Sequence
  Synthetic Peptide
YYYYYHYDYHYDYHYD

SEQ ID NO: 374 - protein, 16 aa, Artificial Sequence
  Synthetic Peptide
YYYYYHYHYHYHYHYH

SEQ ID NO: 375 - protein, 16 aa, Artificial Sequence
  Synthetic Peptide
YYYYYHYDYDYHYDYD

SEQ ID NO: 376 - protein, 16 aa, Artificial Sequence
  Synthetic Peptide
YYYYYHYEYEYHYEYE

SEQ ID NO: 377 - protein, 16 aa, Artificial Sequence
  Synthetic Peptide
NNNNNRNDNRNDNRND

SEQ ID NO: 378 - protein, 16 aa, Artificial Sequence
  Synthetic Peptide
NNNNNRNRNDNDNRNR

SEQ ID NO: 379 - protein, 16 aa, Artificial Sequencev
  Synthetic Peptide
NNNNNENKNENKNENK

SEQ ID NO: 380 - protein, 16 aa, Artificial Sequence
  Synthetic Peptide
NNNNNENENKNKNENE

SEQ ID NO: 381 - protein, 16 aa, Artificial Sequence
  Synthetic Peptide
NNNNNRNENRNENRNE

SEQ ID NO: 382 - protein, 16 aa, Artificial Sequence
  Synthetic Peptide
NNNNNRNRNENENRNE

SEQ ID NO: 383 - protein, 16 aa, Artificial Sequence
  Synthetic Peptide
NNNNNKNDNKNDNKND

SEQ ID NO: 384 - protein, 16 aa, Artificial Sequence
  Synthetic Peptide
NNNNNENHNENHNENH

SEQ ID NO: 385 - protein, 16 aa, Artificial Sequence
  Synthetic Peptide
NNNNNENENHNHNENE

SEQ ID NO: 386 - protein, 16 aa, Artificial Sequence
  Synthetic Peptide
NNNNNRNRNRNRNRNR

SEQ ID NO: 387 - protein, 16 aa, Artificial Sequence
  Synthetic Peptide
NNNNNRNRNRNRNDND

SEQ ID NO: 388 - protein, 16 aa, Artificial Sequence
  Synthetic Peptide
NNNNNRNRNRNDNDND

SEQ ID NO: 389 - protein, 16 aa, Artificial Sequence
  Synthetic Peptide
NNNNNHNDNHNDNHND

SEQ ID NO: 390 - protein, 16 aa, Artificial Sequence
  Synthetic Peptide
NNNNNHNHNHNHNHNH

SEQ ID NO: 391 - protein, 16 aa, Artificial Sequence
  Synthetic Peptide
NNNNNHNDNDNHNDND

SEQ ID NO: 392 - protein, 16 aa, Artificial Sequence
  Synthetic Peptide
NNNNNHNENENHNENE

SEQ ID NO: 393 - protein, 16 aa, Artificial Sequence
  Synthetic Peptide
QQQQQRQDQRQDQRQD

SEQ ID NO: 394 - protein, 16 aa, Artificial Sequence
  Synthetic Peptide
QQQQQRQRQDQDQRQR

SEQ ID NO: 395 - protein, 16 aa, Artificial Sequence
  Synthetic Peptide
QQQQQEQKQEQKQEQK

SEQ ID NO: 396 - protein, 16 aa, Artificial Sequence
  Synthetic Peptide
QQQQQEQEQKQKQEQE

SEQ ID NO: 397 - protein, 16 aa, Artificial Sequence
  Synthetic Peptide
QQQQQRQEQRQEQRQE

SEQ ID NO: 398 - protein, 16 aa, Artificial Sequence
  Synthetic Peptide
QQQQQRQRQEQEQRQE

SEQ ID NO: 399 - protein, 16 aa, Artificial Sequence
  Synthetic Peptide
QQQQQKQDQKQDQKQD

SEQ ID NO: 400 - protein, 16 aa, Artificial Sequence
  Synthetic Peptide
QQQQQEQHQEQHQEQH

SEQ ID NO: 401 - protein, 16 aa, Artificial Sequence
  Synthetic Peptide
QQQQQEQEQHQHQEQE

SEQ ID NO: 402 - protein, 16 aa, Artificial Sequence
  Synthetic Peptide
QQQQQRQRQRQRQRQR

SEQ ID NO: 403 - protein, 16 aa, Artificial Sequence
  Synthetic Peptide
QQQQQRQRQRQRQDQD

SEQ ID NO: 404 - protein, 16 aa, Artificial Sequence
  Synthetic Peptide
QQQQQRQRQRQDQDQD

SEQ ID NO: 405 - protein, 16 aa, Artificial Sequence
  Synthetic Peptide
QQQQQHQDQHQDQHQD

SEQ ID NO: 406 - protein, 16 aa, Artificial Sequence
  Synthetic Peptide
QQQQQHQHQHQHQHQH

SEQ ID NO: 407 - protein, 16 aa, Artificial Sequence
  Synthetic Peptide
QQQQQHQDQDQHQDQD

SEQ ID NO: 408 - protein, 16 aa, Artificial Sequence
  Synthetic Peptide
QQQQQHQEQEQHQEQE

SEQ ID NO: 409 - protein, 8 aa, Artificial Sequence
  Synthetic Peptide
  MISC_FEATURE (1)..(1): Pyridoxamine phosphate modification
  MISC_FEATURE (1)..(1): Methylation
  Xaa (7)..(7): Xaa = ornithine
  NH2 (8)..(8): C-terminal amine
YITNCPXY

SEQ ID NO: 410 - protein, 7 aa, Artificial Sequence
  Synthetic Peptide
  MISC_FEATURE (1)..(1): 3-mercaptopropionyl modification
YFQNCPR

SEQ ID NO: 411 - protein, 9 aa, Artificial Sequence
  Synthetic Peptide
  NH2 (9)..(9): C-terminal amine
CYFQNCPRG

SEQ ID NO: 412 - protein, 8 aa, Artificial Sequence
  Synthetic Peptide
CYFQNCPR

SEQ ID NO: 413 - protein, 4 aa, Artificial Sequence
  Synthetic Peptide
  CONH2 (4)..(4): C-terminal amide
RARA

SEQ ID NO: 414 - protein, 8 aa, Artificial Sequence
  Synthetic Peptide
  CONH2 (8)..(8): C-terminal amide
EARAEARA

SEQ ID NO: 415 - protein, 12 aa, Artificial Sequence
  Synthetic Peptide
RARARADADADA

SEQ ID NO: 416 - protein, 16 aa, Artificial Sequence
  Synthetic Peptide
RARARARADADADADA

SEQ ID NO: 417 - protein, 8 aa, Artificial Sequence
  Synthetic Peptide
RRRRDDDD

SEQ ID NO: 418 - protein, 8 aa, Artificial Sequence
  Synthetic Peptide
GGGGSSSS

SEQ ID NO: 419 - protein, 4 aa, Artificial Sequence
  Synthetic Peptide
KKKK

SEQ ID NO: 420 - protein, 4 aa, Artificial Sequence
  Synthetic Peptide
RRRR

SEQ ID NO: 421 - protein, 4 aa, Artificial Sequence
  Synthetic Peptide
HHHH

SEQ ID NO: 422 - protein, 4 aa, Artificial Sequence
  Synthetic Peptide
DDDD

SEQ ID NO: 423 - protein, 4 aa, Artificial Sequence
  Synthetic Peptide
EEEE

SEQ ID NO: 424 - protein, 4 aa, Artificial Sequence
  Synthetic Peptide
GQGQ

SEQ ID NO: 425 - protein, 6 aa, Artificial Sequence
  Synthetic Peptide
GGQQGG

SEQ ID NO: 426 - protein, 7 aa, Artificial Sequence
  Synthetic Peptide
GQQGQQG

SEQ ID NO: 427 - protein, 8 aa, Artificial Sequence
  Synthetic Peptide
GGQGGQGG

SEQ ID NO: 428 - protein, 16 aa, Artificial Sequence
  Synthetic Peptide
  Xaa (2)..(2): Xaa = beta alanine
  Xaa (4)..(4): Xaa = beta alanine
  Xaa (6)..(6): Xaa = beta alanine
  Xaa (8)..(8): Xaa = beta alanine
  Xaa (10)..(10): Xaa = beta alanine
  Xaa (12)..(12): Xaa = beta alanine
  Xaa (14)..(14): Xaa = beta alanine
  Xaa (16)..(16): Xaa = beta alanine
EXKXEXKXEXKXEXKX

SEQ ID NO: 429 - protein, 8 aa, Artificial Sequence
  Synthetic Peptide
  Xaa (2)..(2): Xaa = beta alanine
  Xaa (4)..(4): Xaa = beta alanine
  Xaa (6)..(6): Xaa = beta alanine
  Xaa (8)..(8): Xaa = beta alanine
EXKXEXKX

SEQ ID NO: 430 - protein, 16 aa, Artificial Sequence
  Synthetic Peptide
  Xaa (2)..(2): Xaa = beta alanine
  Xaa (4)..(4): Xaa = beta alanine
  Xaa (6)..(6): Xaa = beta alanine
  Xaa (8)..(8): Xaa = beta alanine
  Xaa (10)..(10): Xaa = beta alanine
  Xaa (12)..(12): Xaa = beta alanine
  Xaa (14)..(14): Xaa = beta alanine
  Xaa (16)..(16): Xaa = beta alanine
RXDXRXDXRXDXRXDX

SEQ ID NO: 431 - protein, 8 aa, Artificial Sequence
  Synthetic Peptide
  Xaa (2)..(2): Xaa = beta alanine
  Xaa (4)..(4): Xaa = beta alanine
  Xaa (6)..(6): Xaa = beta alanine
  Xaa (8)..(8): Xaa = beta alanine
RXDXRXDX

SEQ ID NO: 432 - protein, 23 aa, Artificial Sequence
  Synthetic Peptide
MSCRAMMEARAEARAEARAEARA

SEQ ID NO: 433 - protein, 16 aa, Artificial Sequence
  Synthetic Peptide
  CONH2 (16)..(16): C-terminal amide
RADARADARADARADA

SEQ ID NO: 434 - protein, 16 aa, Artificial Sequence
  Synthetic Peptide
  MISC_FEATURE (1)..(1): Cy5.5 modification
  CONH2 (16)..(16): C-terminal amide
RADARADARADARADA

SEQ ID NO: 435 - protein, 4 aa, Artificial Sequence
  Synthetic Peptide
  MISC_FEATURE (1)..(1): Cy5.5 modification
  CONH2 (4)..(4): C-terminal amide
EARA

SEQ ID NO: 436 - protein, 4 aa, Artificial Sequence
  Synthetic Peptide
  MISC_FEATURE (1)..(1): Cy5.5 modification
EARA

SEQ ID NO: 437 - protein, 4 aa, Artificial Sequence
  Synthetic Peptide
  MISC_FEATURE (1)..(1): Cy5.5 modification
  CONH2 (4)..(4): C-terminal amide
RARA

SEQ ID NO: 438 - protein, 4 aa, Artificial Sequence
  Synthetic Peptide
  MISC_FEATURE (1)..(1): Cy5.5 modification
RARA

SEQ ID NO: 439 - protein, 8 aa, Artificial Sequence
  Synthetic Peptide
  MISC_FEATURE (1)..(1): Cy5.5 modification
  CONH2 (8)..(8): C-terminal amide
EARAEARA

SEQ ID NO: 440 - protein, 8 aa, Artificial Sequence
  Synthetic Peptide
  MISC_FEATURE (1)..(1): Cy5.5 modification
EARAEARA

SEQ ID NO: 441 - protein, 8 aa, Artificial Sequence
  Synthetic Peptide
  MISC_FEATURE (1)..(1): Cy5.5 modification
  CONH2 (8)..(8): C-terminal amide
RARARARA

SEQ ID NO: 442 - protein, 4 aa, Artificial Sequence
  Synthetic Peptide
  MISC_FEATURE (1)..(1): Cy5.5 modification
RADA

SEQ ID NO: 443 - protein, 4 aa, Artificial Sequence
  Synthetic Peptide
  MISC_FEATURE (1)..(1): Cy5.5 modification
  CONH2 (4)..(4): C-terminal amide
RADA

SEQ ID NO: 444 - protein, 8 aa, Artificial Sequence
  Synthetic Peptide
  MISC_FEATURE (1)..(1): Cy5.5 modification
RADARADA

SEQ ID NO: 445 - protein, 8 aa, Artificial Sequence
  Synthetic Peptide
  MISC_FEATURE (1)..(1): Cy5.5 modification
  CONH2 (4)..(4): C-terminal amide
RADARADA